European Patent Specification EP 3 765 619 B1, published October 9, 2024. Title: INHIBITORS OF MICRO-RNA 22. Applicant: BETH ISRAEL DEACONESS MEDICAL CENTER AALBORG UNIVERSITY. The sequence listing filed with the application follows.

SEQUENCE LISTING (15 sequences)

SEQ ID NO: 1 - RNA, 22 nt, Homo sapiens
aagcugccaguugaagaacugu

SEQ ID NO: 2 - skipped

SEQ ID NO: 3 - DNA, 15 bp, Artificial Sequence
  Synthetic Nucleic Acid
cttcaactggcagct

SEQ ID NO: 4 - DNA, 16 bp, Artificial Sequence
  Synthetic Nucleic Acid
tcttcaactggcagct

SEQ ID NO: 5 - DNA, 17 bp, Artificial Sequence
  Synthetic Nucleic Acid
ttcttcaactggcagct

SEQ ID NO: 6 - DNA, 18 bp, Artificial Sequence
  Synthetic Nucleic Acid
gttcttcaactggcagct

SEQ ID NO: 7 - DNA, 15 bp, Artificial Sequence
  Synthetic Nucleic Acid
cttcaactggcagct

SEQ ID NO: 8 - DNA, 15 bp, Artificial Sequence
  Synthetic Nucleic Acid
cttcaactggcagct

SEQ ID NO: 9 - DNA, 16 bp, Artificial Sequence
  Synthetic Nucleic Acid
tcttcaactggcagct

SEQ ID NO: 10 - DNA, 16 bp, Artificial Sequence
  Synthetic Nucleic Acid
tcttcaactggcagct

SEQ ID NO: 11 - DNA, 16 bp, Artificial Sequence
  Synthetic Nucleic Acid
tcttcaactggcagct

SEQ ID NO: 12 - DNA, 17 bp, Artificial Sequence
  Synthetic Nucleic Acid
ttcttcaactggcagct

SEQ ID NO: 13 - DNA, 18 bp, Artificial Sequence
  Synthetic Nucleic Acid
gttcttcaactggcagct

SEQ ID NO: 14 - DNA, 16 bp, Artificial Sequence
  Synthetic Nucleic Acid
cgaatagttagtagcg

SEQ ID NO: 15 - DNA, 16 bp, Artificial Sequence
  Synthetic Nucleic Acid
cgaatagttagtagcg